European Patent Application EP 4 800 026 A1, published September 2, 2026. Title: ANTIMICROBIAL PEPTIDE VARIANTS AND USES THEREOF. Applicant: ANTINBIO, INC. The sequence listing filed with the application follows.

SEQUENCE LISTING (23 sequences)

SEQ ID NO: 1 - protein, 38 aa, synthetic construct
GFGCTIWGGNDKPCHRHCKSIKGYKGGYCKVGGVCKCY

SEQ ID NO: 2 - protein, 38 aa, synthetic construct
GFGCTIWGGNDDPCHRHCKSIKGYKGGYCKVGGVCKCY

SEQ ID NO: 3 - protein, 38 aa, synthetic construct
GFGCTIWGGNDEPCHRHCKSIKGYKGGYCKVGGVCKCY

SEQ ID NO: 4 - protein, 38 aa, synthetic construct
GFGCTIWGGNDEPCHRHCKSIKGYKGGYCKVGGICKCY

SEQ ID NO: 5 - protein, 38 aa, synthetic construct
GFGCTIWGGNDEPCHRHCKSIKGYKGGYCKFGGVCKCY

SEQ ID NO: 6 - protein, 38 aa, synthetic construct
GFGCTIWGGNDEPCHQHCKSIKGYKGGYCKVGGVCKCY

SEQ ID NO: 7 - protein, 38 aa, synthetic construct
GFGCTIWGGNDEPCHNHCKSIKGYKGGYCKVGGVCKCY

SEQ ID NO: 8 - protein, 38 aa, synthetic construct
GFGCTIWGGNDEPCHRHCKSIKGYKGGYCKFGGICKCY

SEQ ID NO: 9 - protein, 38 aa, synthetic construct
GFGCTIWGGNDEPCHRHCKSIKGYKGGYCKLGGICKCY

SEQ ID NO: 10 - protein, 38 aa, synthetic construct
GFGCTIWGGNDEPCHRHCKSIRGYKGGYCKVGGVCKCY

SEQ ID NO: 11 - protein, 38 aa, synthetic construct
GFGCTIWGGNDEPCHRHCKSIRGYRGGYCKVGGVCKCY

SEQ ID NO: 12 - protein, 38 aa, synthetic construct
GWSCNIWNGNDEPCHQHCKSIRGYRGGYCKFGGVCKCY

SEQ ID NO: 13 - protein, 38 aa, synthetic construct
GWSCNIWNGNDEPCHQHCKSIRGYRGGYCKVGGVCKCY

SEQ ID NO: 14 - protein, 38 aa, synthetic construct
GWSCNIWNGNDEPCHQHCKSIKGYKGGYCKVGGVCKCY

SEQ ID NO: 15 - protein, 38 aa, synthetic construct
GWSCNIWNGNDEPCHRHCKSIKGYKGGYCKVGGVCKCY

SEQ ID NO: 16 - protein, 38 aa, synthetic construct
GWSCNIWNGNDEPCHNHCKSIKGYKGGYCKVGGVCKCY

SEQ ID NO: 17 - protein, 38 aa, synthetic construct
GWSCNIWNGNDEPCHRHCKSIKGYKGGYCKFGGICKCY

SEQ ID NO: 18 - protein, 38 aa, synthetic construct
GWSCNIWNGNDEPCHKHCKSIRGYRGGYCKFGGICKCY

SEQ ID NO: 19 - protein, 38 aa, synthetic construct
GWSCNIWNEDDLRCHNHCKSIRGYRGGYCKFGGICKCY

SEQ ID NO: 20 - protein, 38 aa, synthetic construct
GWSCNIWNEDDLRCHQHCKSIKGYKGGYCKVGGVCKCY

SEQ ID NO: 21 - protein, 38 aa, synthetic construct
GWSCGFFGGNDEPCHQHCKSIRGYRGGYCKVGGICKCY

SEQ ID NO: 22 - protein, 38 aa, synthetic construct
  VARIANT 2: note = F or W
  VARIANT 3: note = G or S
  VARIANT 5: note = T, N or G
  VARIANT 6: note = I or F
  VARIANT 7: note = W or F
  VARIANT 8: note = G or N
  VARIANT 9: note = G or E
  VARIANT 10: note = N or D
  VARIANT 12: note = E, L, or D
  VARIANT 13: note = P or R
  VARIANT 16: note = R, Q, N, or K
  VARIANT 22: note = K or R
  VARIANT 25: note = K or R
  VARIANT 31: note = V, F, or L
  VARIANT 34: note = V or I
GXXCXXXXXXDXXCHXHCKSIXGYXGGYCKXGGXCKCY

SEQ ID NO: 23 - protein, 38 aa, synthetic construct
  VARIANT 2: note = F or W
  VARIANT 3: note = G or S
  VARIANT 5: note = T, N or G
  VARIANT 6: note = I or F
  VARIANT 7: note = W or F
  VARIANT 12: note = E, L, or D
  VARIANT 13: note = P or R
  VARIANT 16: note = R, Q, N, or K
  VARIANT 22: note = K or R
  VARIANT 25: note = K or R
  VARIANT 31: note = V, F, or L
  VARIANT 34: note = V or I
GXXCXXXGGNDXXCHXHCKSIXGYXGGYCKXGGXCKCY